European Patent Application EP 4 386 006 A1, published June 19, 2024. Title: 抗体药物偶联物及其应用. Applicant: 江苏康宁杰瑞生物制药有限公司. The sequence listing filed with the application follows.

SEQUENCE LISTING (57 sequences)

SEQ ID NO: 1 - protein, 8 aa, synthetic construct
  REGION 1..8: note = Trastuzumab LCDR1
QDVNTAVA

SEQ ID NO: 2 - protein, 7 aa, synthetic construct
  REGION 1..7: note = Trastuzumab LCDR2
SASFLYS

SEQ ID NO: 3 - protein, 9 aa, synthetic construct
  REGION 1..9: note = Trastuzumab LCDR3
QQHYTTPPT

SEQ ID NO: 4 - protein, 8 aa, synthetic construct
  REGION 1..8: note = Pertuzumab LCDR1
QDVSIGVA

SEQ ID NO: 5 - protein, 7 aa, synthetic construct
  REGION 1..7: note = Pertuzumab LCDR2
SASYRYT

SEQ ID NO: 6 - protein, 9 aa, synthetic construct
  REGION 1..9: note = Pertuzumab LCDR3
QQYYIYPYT

SEQ ID NO: 7 - protein, 107 aa, synthetic construct [sequence omitted]

SEQ ID NO: 8 - protein, 107 aa, synthetic construct
  REGION 1..107: note = VL2
DIQMTQSPSSLSASVGDRVTITCRASQDVNIAVAWYQQKPGKAPKLLIYSASFLYSGVPSRFSGSRSGTDFTLTISSLQPEDFATYYCQQHYTTPPTFGQGTKVEIK

SEQ ID NO: 9 - protein, 107 aa, synthetic construct
  REGION 1..107: note = VL3
DIQMTQSPSSLSASVGDRVTITCRASQDVNTAVAWYQQKPGKAPKLLIYSASFLYSGVPSRFSGSRSGTDFTLTISSLQPEDFATYYCQQHYTYPPTFGQGTKVEIK

SEQ ID NO: 10 - protein, 107 aa, synthetic construct
  REGION 1..107: note = VL4
DIQMTQSPSSLSASVGDRVTITCRASQDVNIAVAWYQQKPGKAPKLLIYSASFLYSGVPSRFSGSRSGTDFTLTISSLQPEDFATYYCQQHYTYPPTFGQGTKVEIK

SEQ ID NO: 11 - protein, 107 aa, synthetic construct [sequence omitted]

SEQ ID NO: 12 - protein, 107 aa, synthetic construct
  REGION 1..107: note = VL6
DIQMTQSPSSLSASVGDRVTITCKASQDVSIGVAWYQQKPGKAPKLLIYSASYRYTGVPSRFSGSGSGTDFTLTISSLQPEDFATYYCQQYYITPYTFGQGTKVEIK

SEQ ID NO: 13 - protein, 214 aa, synthetic construct
  REGION 1..214: note = LC1
DIQMTQSPSSLSASVGDRVTITCRASQDVNTAVAWYQQKPGKAPKLLIYSASFLYSGVPSRFSGSRSGTDFTLTISSLQPEDFATYYCQQHYTTPPTFGQGTKVEIKRTVAAPSVFIFPPSDEQLKSGTASVVCLLNNFYPREAKVQWKVDNALQSGNSQESVTEQDSKDSTYSLSSTLTLSKADYEKHKVYACEVTHQGLSSPVTKSFNRGEC

SEQ ID NO: 14 - protein, 214 aa, synthetic construct
  REGION 1..214: note = LC2
DIQMTQSPSSLSASVGDRVTITCRASQDVNIAVAWYQQKPGKAPKLLIYSASFLYSGVPSRFSGSRSGTDFTLTISSLQPEDFATYYCQQHYTTPPTFGQGTKVEIKRTVAAPSVFIFPPSDEQLKSGTASVVCLLNNFYPREAKVQWKVDNALQSGNSQESVTEQDSKDSTYSLSSTLTLSKADYEKHKVYACEVTHQGLSSPVTKSFNRGEC

SEQ ID NO: 15 - protein, 214 aa, synthetic construct
  REGION 1..214: note = LC3
DIQMTQSPSSLSASVGDRVTITCRASQDVNTAVAWYQQKPGKAPKLLIYSASFLYSGVPSRFSGSRSGTDFTLTISSLQPEDFATYYCQQHYTYPPTFGQGTKVEIKRTVAAPSVFIFPPSDEQLKSGTASVVCLLNNFYPREAKVQWKVDNALQSGNSQESVTEQDSKDSTYSLSSTLTLSKADYEKHKVYACEVTHQGLSSPVTKSFNRGEC

SEQ ID NO: 16 - protein, 214 aa, synthetic construct
  REGION 1..214: note = LC4
DIQMTQSPSSLSASVGDRVTITCRASQDVNIAVAWYQQKPGKAPKLLIYSASFLYSGVPSRFSGSRSGTDFTLTISSLQPEDFATYYCQQHYTYPPTFGQGTKVEIKRTVAAPSVFIFPPSDEQLKSGTASVVCLLNNFYPREAKVQWKVDNALQSGNSQESVTEQDSKDSTYSLSSTLTLSKADYEKHKVYACEVTHQGLSSPVTKSFNRGEC

SEQ ID NO: 17 - protein, 214 aa, synthetic construct
  REGION 1..214: note = LC5
DIQMTQSPSSLSASVGDRVTITCKASQDVSIGVAWYQQKPGKAPKLLIYSASYRYTGVPSRFSGSGSGTDFTLTISSLQPEDFATYYCQQYYIYPYTFGQGTKVEIKRTVAAPSVFIFPPSDEQLKSGTASVVCLLNNFYPREAKVQWKVDNALQSGNSQESVTEQDSKDSTYSLSSTLTLSKADYEKHKVYACEVTHQGLSSPVTKSFNRGEC

SEQ ID NO: 18 - protein, 214 aa, synthetic construct
  REGION 1..214: note = LC6
DIQMTQSPSSLSASVGDRVTITCKASQDVSIGVAWYQQKPGKAPKLLIYSASYRYTGVPSRFSGSGSGTDFTLTISSLQPEDFATYYCQQYYITPYTFGQGTKVEIKRTVAAPSVFIFPPSDEQLKSGTASVVCLLNNFYPREAKVQWKVDNALQSGNSQESVTEQDSKDSTYSLSSTLTLSKADYEKHKVYACEVTHQGLSSPVTKSFNRGEC

SEQ ID NO: 19 - protein, 119 aa, synthetic construct [sequence omitted]

SEQ ID NO: 20 - protein, 120 aa, synthetic construct [sequence omitted]

SEQ ID NO: 21 - protein, 449 aa, synthetic construct
  REGION 1..449: note = HC1
EVQLVESGGGLVQPGGSLRLSCAASGFTFTDYTMDWVRQAPGKGLEWVADVNPNSGGSIYNQRFKGRFTLSVDRSKNTLYLQMNSLRAEDTAVYYCARNLGPSFYFDYWGQGTLVTVSSASTKGPSVFPLAPSSKSTSGGTAALGCLVKDYFPEPVTVSWNSGALTSGVHTFPAVLQSSGLYSLSSVVTVPSSSLGTQTYICNVNHKPSNTKVDKKVEPKSCDKTHTCPPCPAPELLGGPSVFLFPPKPKDTLMISRTPEVTCVVVDVSHEDPEVKFNWYVDGVEVHNAKTKPREEQYNSTYRVVSVLTVLHQDWLNGKEYKCKVSNKALPAPIEKTISKAKGQPREPQVYTLPPSRDELTKNQVSLWCLVKGFYPSDIAVEWESNGQPENNYKTTPPVLDSDGSFFLYSALTVDKSRWQQGNVFSCSVMHEALHNHYTQKSLSLSPGK

SEQ ID NO: 22 - protein, 450 aa, synthetic construct
  REGION 1..450: note = HC2
EVQLVESGGGLVQPGGSLRLSCAASGFNIKDTYIHWVRQAPGKGLEWVARIYPTNGYTRYADSVKGRFTISADTSKNTAYLQMNSLRAEDTAVYYCSRWGGDGFYAMDYWGQGTLVTVSSASTKGPSVFPLAPSSKSTSGGTAALGCLVKDYFPEPVTVSWNSGALTSGVHTFPAVLQSSGLYSLSSVVTVPSSSLGTQTYICNVNHKPSNTKVDKKVEPKSCDKTHTCPPCPAPELLGGPSVFLFPPKPKDTLMISRTPEVTCVVVDVSHEDPEVKFNWYVDGVEVHNAKTKPREEQYNSTYRVVSVLTVLHQDWLNGKEYKCKVSNKALPAPIEKTISKAKGQPREPQVYTLPPSRDELTKNQVSLSCAVKGFYPSDIAVEWESNGQPENNYKTTPPVLDSDGSFKLVSKLTVDKSRWQQGNVFSCSVMHEALHNHYTQKSLSLSPGK

SEQ ID NO: 23 - protein, 450 aa, synthetic construct
  REGION 1..450: note = HC3
EVQLVESGGGLVQPGGSLRLSCAASGFNIKDTYIHWVRQAPGKGLEWVARIYPTNGYTRYADSVKGRFTISADTSKNTAYLQMNSLRAEDTAVYYCSRWGGDGFYAMDYWGQGTLVTVSSASTKGPSVFPLAPSSKSTSGGTAALGCLVKDYFPEPVTVSWNSGALTSGVHTFPAVLQSSGLYSLSSVVTVPSSSLGTQTYICNVNHKPSNTKVDKKVEPKSCDKTHTCPPCPAPELLGGPSVFLFPPKPKDTLMISRTPEVTCVVVDVSHEDPEVKFNWYVDGVEVHNAKTKPREEQYNSTYRVVSVLTVLHQDWLNGKEYKCKVSNKALPAPIEKTISKAKGQPREPQVYTLPPCRDELTKNQVSLWCLVKGFYPSDIAVEWESNGQPENNYKTTPPVLDSDGSFFLYSKLTVDKSRWQQGNVFSCSVMHEALHNHYTQKSLSLSPGK

SEQ ID NO: 24 - protein, 449 aa, synthetic construct
  REGION 1..449: note = HC4
EVQLVESGGGLVQPGGSLRLSCAASGFTFTDYTMDWVRQAPGKGLEWVADVNPNSGGSIYNQRFKGRFTLSVDRSKNTLYLQMNSLRAEDTAVYYCARNLGPSFYFDYWGQGTLVTVSSASTKGPSVFPLAPSSKSTSGGTAALGCLVKDYFPEPVTVSWNSGALTSGVHTFPAVLQSSGLYSLSSVVTVPSSSLGTQTYICNVNHKPSNTKVDKKVEPKSCDKTHTCPPCPAPELLGGPSVFLFPPKPKDTLMISRTPEVTCVVVDVSHEDPEVKFNWYVDGVEVHNAKTKPREEQYNSTYRVVSVLTVLHQDWLNGKEYKCKVSNKALPAPIEKTISKAKGQPREPQVCTLPPSRDELTKNQVSLSCAVKGFYPSDIAVEWESNGQPENNYKTTPPVLDSDGSFFLVSKLTVDKSRWQQGNVFSCSVMHEALHNHYTQKSLSLSPGK

SEQ ID NO: 25 - protein, 330 aa, synthetic construct
  REGION 1..330: note = FC1
ASTKGPSVFPLAPSSKSTSGGTAALGCLVKDYFPEPVTVSWNSGALTSGVHTFPAVLQSSGLYSLSSVVTVPSSSLGTQTYICNVNHKPSNTKVDKKVEPKSCDKTHTCPPCPAPELLGGPSVFLFPPKPKDTLMISRTPEVTCVVVDVSHEDPEVKFNWYVDGVEVHNAKTKPREEQYNSTYRVVSVLTVLHQDWLNGKEYKCKVSNKALPAPIEKTISKAKGQPREPQVYTLPPSRDELTKNQVSLWCLVKGFYPSDIAVEWESNGQPENNYKTTPPVLDSDGSFFLYSALTVDKSRWQQGNVFSCSVMHEALHNHYTQKSLSLSPGK

SEQ ID NO: 26 - protein, 330 aa, synthetic construct
  REGION 1..330: note = FC2
ASTKGPSVFPLAPSSKSTSGGTAALGCLVKDYFPEPVTVSWNSGALTSGVHTFPAVLQSSGLYSLSSVVTVPSSSLGTQTYICNVNHKPSNTKVDKKVEPKSCDKTHTCPPCPAPELLGGPSVFLFPPKPKDTLMISRTPEVTCVVVDVSHEDPEVKFNWYVDGVEVHNAKTKPREEQYNSTYRVVSVLTVLHQDWLNGKEYKCKVSNKALPAPIEKTISKAKGQPREPQVYTLPPSRDELTKNQVSLSCAVKGFYPSDIAVEWESNGQPENNYKTTPPVLDSDGSFKLVSKLTVDKSRWQQGNVFSCSVMHEALHNHYTQKSLSLSPGK

SEQ ID NO: 27 - protein, 471 aa, synthetic construct
  REGION 1..471: note = FC3
EVQLLESGGGVVQPGRSLRLSCIASGFTFSSYPMTWVRQAPGKGLEWVASISYDGSYKYKADSMKGRLTISRDNSKNTLYLEMNSLTAEDTAVYYCARTAFFNAYDFWGQGTLVTVSSASTKGPSVGGGGSGGGGSEIVMTQSPATLSVSPGERATLSCRASQSVRSNLAWYQQKPGQAPRLLIYAASTRATGIPARFSGSGSGTEFTLTISSLQSEDFAVYYCQQYNEWFRTSGQGTKVEIKRDKTHTCPPCPAPELLGGPSVFLFPPKPKDTLMISRTPEVTCVVVDVSHENPEVKFNWYVDGVEVHNAKTKPREEQYNSTYRVVSVLTVLHQDWLNGKEYKCKVSNKALPAPIEKTISKAKGQPREPQVCTLPPSRDELTKNQVSLWCLVKGFYPSDIAVEWESNGQPENNYKTTPPVLDSDGSFFLYSKLTVDKSRWQQGNVFSCSVMHEALHNHYTQKSLSLSPGK

SEQ ID NO: 28 - protein, 227 aa, synthetic construct
  REGION 1..227: note = FC4
DKTHTCPPCPAPELLGGPSVFLFPPKPKDTLMISRTPEVTCVVVDVSHEDPEVKFNWYVDGVEVHNAKTKPREEQYNSTYRVVSVLTVLHQDWLNGKEYKCKVSNKALPAPIEKTISKAKGQPREPQVYTLPPSRCELTKNQVSLSCAVKGFYPSDIAVEWESNGQPENNYKTTPPVLDSDGSFFLVSKLTVDKSRWQQGNVFSCSVMHEALHNHYTQKSLSLSPGK

SEQ ID NO: 29 - protein, 227 aa, synthetic construct
  REGION 1..227: note = FC5
DKTHTCPPCPAPELLGGPSVFLFPPKPKDTLMISRTPEVTCVVVDVSHEDPEVKFNWYVDGVEVHNAKTKPREEQYNSTYRVVSVLTVLHQDWLNGKEYKCKVSNKALPAPIEKTISKAKGQPREPQVYTLPPSRCELTKNQVSLSCAVKGFYPSDIAVEWESNGQPENNYKTTPPVLDSDGSFKLVSKLTVDKSRWQQGNVFSCSVMHEALHNHYTQKSLSLSPGK

SEQ ID NO: 30 - protein, 471 aa, synthetic construct
  REGION 1..471: note = FC6
EVQLLESGGGVVQPGRSLRLSCIASGFTFSSYPMTWVRQAPGKGLEWVASISYDGSYKYKADSMKGRLTISRDNSKNTLYLEMNSLTAEDTAVYYCARTAFFNAYDFWGQGTLVTVSSASTKGPSVGGGGSGGGGSEIVMTQSPATLSVSPGERATLSCRASQSVRSNLAWYQQKPGQAPRLLIYAASTRATGIPARFSGSGSGTEFTLTISSLQSEDFAVYYCQQYNEWFRTSGQGTKVEIKRDKTHTCPPCPAPELLGGPSVFLFPPKPKDTLMISRTPEVTCVVVDVSHENPEVKFNWYVDGVEVHNAKTKPREEQYNSTYRVVSVLTVLHQDWLNGKEYKCKVSNKALPAPIEKTISKAKGQPREPQVCTLPPSRDELTKNQVSLWCLVKGFYPSDIAVEWESNGQPENNYKTTPPVLDSDGSFKLYSKLTVDKSRWQQGNVFSCSVMHEALHNHYTQKSLSLSPGK

SEQ ID NO: 31 - protein, 471 aa, synthetic construct
  REGION 1..471: note = FC7
EVQLLESGGGVVQPGRSLRLSCIASGFTFSSYPMTWVRQAPGKGLEWVASISYDGSYKYKADSMKGRLTISRDNSKNTLYLEMNSLTAEDTAVYYCARTAFFNAYDFWGQGTLVTVSSASTKGPSVGGGGSGGGGSEIVMTQSPATLSVSPGERATLSCRASQSVRSNLAWYQQKPGQAPRLLIYAASTRATGIPARFSGSGSGTEFTLTISSLQSEDFAVYYCQQYNEWFRTSGQGTKVEIKRDKTHTCPPCPAPELLGGPSVFLFPPKPKDTLMISRTPEVTCVVVDVSHENPEVKFNWYVDGVEVHNAKTKPREEQYNSTYRVVSVLTVLHQDWLNGKEYKCKVSNKALPAPIEKTISKAKGQPREPQVCTLPPSRDELTKNQVSLWCLVKGFYPSDIAVEWESNGQPENNYKTTPPVLDSDGSFFLYSELTVDKSRWQQGNVFSCSVMHEALHNHYTQKSLSLSPGK

SEQ ID NO: 32 - protein, 471 aa, synthetic construct
  REGION 1..471: note = FC8
EVQLLESGGGVVQPGRSLRLSCIASGFTFSSYPMTWVRQAPGKGLEWVASISYDGSYKYKADSMKGRLTISRDNSKNTLYLEMNSLTAEDTAVYYCARTAFFNAYDFWGQGTLVTVSSASTKGPSVGGGGSGGGGSEIVMTQSPATLSVSPGERATLSCRASQSVRSNLAWYQQKPGQAPRLLIYAASTRATGIPARFSGSGSGTEFTLTISSLQSEDFAVYYCQQYNEWFRTSGQGTKVEIKRDKTHTCPPCPAPELLGGPSVFLFPPKPKDTLMISRTPEVTCVVVDVSHENPEVKFNWYVDGVEVHNAKTKPREEQYNSTYRVVSVLTVLHQDWLNGKEYKCKVSNKALPAPIEKTISKAKGQPREPQVCTLPPSRDELTKNQVSLWCLVKGFYPSDIAVEWESNGQPENNYKTTPPVLDSDGSFFLYSALTVDKSRWQQGNVFSCSVMHEALHNHYTQKSLSLSPGK

SEQ ID NO: 33 - protein, 471 aa, synthetic construct
  REGION 1..471: note = FC9
EVQLLESGGGVVQPGRSLRLSCIASGFTFSSYPMTWVRQAPGKGLEWVASISYDGSYKYKADSMKGRLTISRDNSKNTLYLEMNSLTAEDTAVYYCARTAFFNAYDFWGQGTLVTVSSASTKGPSVGGGGSGGGGSEIVMTQSPATLSVSPGERATLSCRASQSVRSNLAWYQQKPGQAPRLLIYAASTRATGIPARFSGSGSGTEFTLTISSLQSEDFAVYYCQQYNEWFRTSGQGTKVEIKRDKTHTCPPCPAPELLGGPSVFLFPPKPKDTLMISRTPEVTCVVVDVSHENPEVKFNWYVDGVEVHNAKTKPREEQYNSTYRVVSVLTVLHQDWLNGKEYKCKVSNKALPAPIEKTISKAKGQPREPEVCTLPPSRDELTENQVSLWCLVKGFYPSDIAVEWESNGQPENNYKTTPPVLDSDGSFKLYSKLTVDKSRWQQGNVFSCSVMHEALHNHYTQKSLSLSPGK

SEQ ID NO: 34 - protein, 227 aa, synthetic construct
  REGION 1..227: note = FC10
DKTHTCPPCPAPELLGGPSVFLFPPKPKDTLMISRTPEVTCVVVDVSHEDPEVKFNWYVDGVEVHNAKTKPREEQYNSTYRVVSVLTVLHQDWLNGKEYKCKVSNKALPAPIEKTISKAKGQPREPRVYTLPPSRCELTKNQVSLSCAVKGFYPSDIAVEWESNGQPENNYKTTPPVLDSDGSFFLVSKLTVDKSRWQQGNVFSCSVMHEALHNHYTQKSLSLSPGK

SEQ ID NO: 35 - protein, 471 aa, synthetic construct
  REGION 1..471: note = FC11
EVQLLESGGGVVQPGRSLRLSCIASGFTFSSYPMTWVRQAPGKGLEWVASISYDGSYKYKADSMKGRLTISRDNSKNTLYLEMNSLTAEDTAVYYCARTAFFNAYDFWGQGTLVTVSSASTKGPSVGGGGSGGGGSEIVMTQSPATLSVSPGERATLSCRASQSVRSNLAWYQQKPGQAPRLLIYAASTRATGIPARFSGSGSGTEFTLTISSLQSEDFAVYYCQQYNEWFRTSGQGTKVEIKRDKTHTCPPCPAPELLGGPSVFLFPPKPKDTLMISRTPEVTCVVVDVSHENPEVKFNWYVDGVEVHNAKTKPREEQYNSTYRVVSVLTVLHQDWLNGKEYKCKVSNKALPAPIEKTISKAKGQPREPRVCTLPPSRDELTKNQVSLWCLVKGFYPSDIAVEWESNGQPENNYKTTPPVLDSDGSFKLYSKLTVDKSRWQQGNVFSCSVMHEALHNHYTQKSLSLSPGK

SEQ ID NO: 36 - protein, 227 aa, synthetic construct
  REGION 1..227: note = FC12
DKTHTCPPCPAPELLGGPSVFLFPPKPKDTLMISRTPEVTCVVVDVSHEDPEVKFNWYVDGVEVHNAKTKPREEQYNSTYRVVSVLTVLHQDWLNGKEYKCKVSNKALPAPIEKTISKAKGQPREPEVYTLPPSRCELTENQVSLSCAVKGFYPSDIAVEWESNGQPENNYKTTPPVLDSDGSFFLVSKLTVDKSRWQQGNVFSCSVMHEALHNHYTQKSLSLSPGK

SEQ ID NO: 37 - protein, 471 aa, synthetic construct
  REGION 1..471: note = FC13
EVQLLESGGGVVQPGRSLRLSCIASGFTFSSYPMTWVRQAPGKGLEWVASISYDGSYKYKADSMKGRLTISRDNSKNTLYLEMNSLTAEDTAVYYCARTAFFNAYDFWGQGTLVTVSSASTKGPSVGGGGSGGGGSEIVMTQSPATLSVSPGERATLSCRASQSVRSNLAWYQQKPGQAPRLLIYAASTRATGIPARFSGSGSGTEFTLTISSLQSEDFAVYYCQQYNEWFRTSGQGTKVEIKRDKTHTCPPCPAPELLGGPSVFLFPPKPKDTLMISRTPEVTCVVVDVSHENPEVKFNWYVDGVEVHNAKTKPREEQYNSTYRVVSVLTVLHQDWLNGKEYKCKVSNKALPAPIEKTISKAKGQPREPEVCTLPPSRDELTENQVSLWCLVKGFYPSDIAVEWESNGQPENNYKTTPPVLDSDGSFFLYSALTVDKSRWQQGNVFSCSVMHEALHNHYTQKSLSLSPGK

SEQ ID NO: 38 - protein, 227 aa, synthetic construct
  REGION 1..227: note = FC14
DKTHTCPPCPAPELLGGPSVFLFPPKPKDTLMISRTPEVTCVVVDVSHEDPEVKFNWYVDGVEVHNAKTKPREEQYNSTYRVVSVLTVLHQDWLNGKEYKCKVSNKALPAPIEKTISKAKGQPREPRVYTLPPSRCELTKNQVSLSCAVKGFYPSDIAVEWESNGQPENNYKTTPPVLDSDGSFKLVSKLTVDKSRWQQGNVFSCSVMHEALHNHYTQKSLSLSPGK

SEQ ID NO: 39 - protein, 471 aa, synthetic construct
  REGION 1..471: note = FC15
EVQLLESGGGVVQPGRSLRLSCIASGFTFSSYPMTWVRQAPGKGLEWVASISYDGSYKYKADSMKGRLTISRDNSKNTLYLEMNSLTAEDTAVYYCARTAFFNAYDFWGQGTLVTVSSASTKGPSVGGGGSGGGGSEIVMTQSPATLSVSPGERATLSCRASQSVRSNLAWYQQKPGQAPRLLIYAASTRATGIPARFSGSGSGTEFTLTISSLQSEDFAVYYCQQYNEWFRTSGQGTKVEIKRDKTHTCPPCPAPELLGGPSVFLFPPKPKDTLMISRTPEVTCVVVDVSHENPEVKFNWYVDGVEVHNAKTKPREEQYNSTYRVVSVLTVLHQDWLNGKEYKCKVSNKALPAPIEKTISKAKGQPREPRVCTLPPSRDELTKNQVSLWCLVKGFYPSDIAVEWESNGQPENNYKTTPPVLDSDGSFFLYSALTVDKSRWQQGNVFSCSVMHEALHNHYTQKSLSLSPGK

SEQ ID NO: 40 - protein, 227 aa, synthetic construct
  REGION 1..227: note = FC16
DKTHTCPPCPAPELLGGPSVFLFPPKPKDTLMISRTPEVTCVVVDVSHEDPEVKFNWYVDGVEVHNAKTKPREEQYNSTYRVVSVLTVLHQDWLNGKEYKCKVSNKALPAPIEKTISKAKGQPREPEVYTLPPSRCELTENQVSLSCAVKGFYPSDIAVEWESNGQPENNYKTTPPVLDSDGSFKLVSKLTVDKSRWQQGNVFSCSVMHEALHNHYTQKSLSLSPGK

SEQ ID NO: 41 - protein, 471 aa, synthetic construct
  REGION 1..471: note = FC17
EVQLLESGGGVVQPGRSLRLSCIASGFTFSSYPMTWVRQAPGKGLEWVASISYDGSYKYKADSMKGRLTISRDNSKNTLYLEMNSLTAEDTAVYYCARTAFFNAYDFWGQGTLVTVSSASTKGPSVGGGGSGGGGSEIVMTQSPATLSVSPGERATLSCRASQSVRSNLAWYQQKPGQAPRLLIYAASTRATGIPARFSGSGSGTEFTLTISSLQSEDFAVYYCQQYNEWFRTSGQGTKVEIKRDKTHTCPPCPAPELLGGPSVFLFPPKPKDTLMISRTPEVTCVVVDVSHENPEVKFNWYVDGVEVHNAKTKPREEQYNSTYRVVSVLTVLHQDWLNGKEYKCKVSNKALPAPIEKTISKAKGQPREPQVCTLPPSRDELTKNQVSLWCEVKGFYPSDIAVEWESNGQPENNYKTTPPVLDSDGSFFLYSALTVDKSRWQQGNVFSCSVMHEALHNHYTQKSLSLSPGK

SEQ ID NO: 42 - protein, 471 aa, synthetic construct
  REGION 1..471: note = FC18
EVQLLESGGGVVQPGRSLRLSCIASGFTFSSYPMTWVRQAPGKGLEWVASISYDGSYKYKADSMKGRLTISRDNSKNTLYLEMNSLTAEDTAVYYCARTAFFNAYDFWGQGTLVTVSSASTKGPSVGGGGSGGGGSEIVMTQSPATLSVSPGERATLSCRASQSVRSNLAWYQQKPGQAPRLLIYAASTRATGIPARFSGSGSGTEFTLTISSLQSEDFAVYYCQQYNEWFRTSGQGTKVEIKRDKTHTCPPCPAPELLGGPSVFLFPPKPKDTLMISRTPEVTCVVVDVSHENPEVKFNWYVDGVEVHNAKTKPREEQYNSTYRVVSVLTVLHQDWLNGKEYKCKVSNKALPAPIEKTISKAKGQPREPQVYTLPPSRDELTKNQVSLWCLVKGFYPSDIAVEWESNGQPENNYDTTPPVLDSDGSFFLYSALTVDKSRWQQGNVFSCSVMHEALHNHYTQKSLSLSPGK

SEQ ID NO: 43 - protein, 227 aa, synthetic construct
  REGION 1..227: note = FC19
DKTHTCPPCPAPELLGGPSVFLFPPKPKDTLMISRTPEVTCVVVDVSHEDPEVKFNWYVDGVEVHNAKTKPREEQYNSTYRVVSVLTVLHQDWLNGKEYKCKVSNKALPAPIEKTISKAKGQPREPQVYTLPPSRDELTKNQVSLSCAVKGFYPSDIAVEWESNGQPENNYKTTPPVLSSDGSFKLVSKLTVDKSRWQQGNVFSCSVMHEALHNHYTQKSLSLSPGK

SEQ ID NO: 44 - protein, 471 aa, synthetic construct
  REGION 1..471: note = FC20
EVQLLESGGGVVQPGRSLRLSCIASGFTFSSYPMTWVRQAPGKGLEWVASISYDGSYKYKADSMKGRLTISRDNSKNTLYLEMNSLTAEDTAVYYCARTAFFNAYDFWGQGTLVTVSSASTKGPSVGGGGSGGGGSEIVMTQSPATLSVSPGERATLSCRASQSVRSNLAWYQQKPGQAPRLLIYAASTRATGIPARFSGSGSGTEFTLTISSLQSEDFAVYYCQQYNEWFRTSGQGTKVEIKRDKTHTCPPCPAPELLGGPSVFLFPPKPKDTLMISRTPEVTCVVVDVSHENPEVKFNWYVDGVEVHNAKTKPREEQYNSTYRVVSVLTVLHQDWLNGKEYKCKVSNKALPAPIEKTISKAKGQPREPQVYTLPPSRDELTKNQVSLWCLVKGFYPSDIAVEWESNGQPENNYKTTPPVLDSDGSFFLYSALTVDKSRWQQGNVFSCSVMHEALHNHYTQKSLSLSPGK

SEQ ID NO: 45 - protein, 227 aa, synthetic construct
  REGION 1..227: note = FC21
DKTHTCPPCPAPELLGGPSVFLFPPKPKDTLMISRTPEVTCVVVDVSHEDPEVKFNWYVDGVEVHNAKTKPREEQYNSTYRVVSVLTVLHQDWLNGKEYKCKVSNKALPAPIEKTISKAKGQPREPQVYTLPPSRDELTKNQVSLSCGVKGFYPSDIAVEWESNGQPENNYKTTPPVLDSDGSFKLASKLTVDKSRWQQGNVFSCSVMHEALHNHYTQKSLSLSPGK

SEQ ID NO: 46 - protein, 227 aa, synthetic construct
  REGION 1..227: note = FC22
DKTHTCPPCPAPELLGGPSVFLFPPKPKDTLMISRTPEVTCVVVDVSHEDPEVKFNWYVDGVEVHNAKTKPREEQYNSTYRVVSVLTVLHQDWLNGKEYKCKVSNKALPAPIEKTISKAKGQPREPQVYTLPPSRDALTKNQVSLSCAVKGFYPSDIAVEWESNGQPENNYKTTPPVLDSDGSFKLVSKLTVDKSRWQQGNVFSCSVMHEALHNHYTQKSLSLSPGK

SEQ ID NO: 47 - protein, 471 aa, synthetic construct
  REGION 1..471: note = FC23
EVQLLESGGGVVQPGRSLRLSCIASGFTFSSYPMTWVRQAPGKGLEWVASISYDGSYKYKADSMKGRLTISRDNSKNTLYLEMNSLTAEDTAVYYCARTAFFNAYDFWGQGTLVTVSSASTKGPSVGGGGSGGGGSEIVMTQSPATLSVSPGERATLSCRASQSVRSNLAWYQQKPGQAPRLLIYAASTRATGIPARFSGSGSGTEFTLTISSLQSEDFAVYYCQQYNEWFRTSGQGTKVEIKRDKTHTCPPCPAPELLGGPSVFLFPPKPKDTLMISRTPEVTCVVVDVSHENPEVKFNWYVDGVEVHNAKTKPREEQYNSTYRVVSVLTVLHQDWLNGKEYKCKVSNKALPAPIEKTISKAKGQPREPQVDTLPPDRDELTKNQVSLWCLVKGFYPSDIAVEWESNGQPENNYKTTPPVLDSDGSFFLYSALTVDKSRWQQGNVFSCSVMHEALHNHYTQKSLSLSPGK

SEQ ID NO: 48 - protein, 471 aa, synthetic construct
  REGION 1..471: note = FC24
EVQLLESGGGVVQPGRSLRLSCIASGFTFSSYPMTWVRQAPGKGLEWVASISYDGSYKYKADSMKGRLTISRDNSKNTLYLEMNSLTAEDTAVYYCARTAFFNAYDFWGQGTLVTVSSASTKGPSVGGGGSGGGGSEIVMTQSPATLSVSPGERATLSCRASQSVRSNLAWYQQKPGQAPRLLIYAASTRATGIPARFSGSGSGTEFTLTISSLQSEDFAVYYCQQYNEWFRTSGQGTKVEIKRDKTHTCPPCPAPELLGGPSVFLFPPKPKDTLMISRTPEVTCVVVDVSHENPEVKFNWYVDGVEVHNAKTKPREEQYNSTYRVVSVLTVLHQDWLNGKEYKCKVSNKALPAPIEKTISKAKGQPREPQVYTLPPSRDELTKNQVSLWCLVKGFYPSDIAVEWESNGQPENNYKTTPPVLDSDGSFKLYSKLTVDKSRWQQGNVFSCSVMHEALHNHYTQKSLSLSPGK

SEQ ID NO: 49 - protein, 227 aa, synthetic construct
  REGION 1..227: note = FC25
DKTHTCPPCPAPELLGGPSVFLFPPKPKDTLMISRTPEVTCVVVDVSHEDPEVKFNWYVDGVEVHNAKTKPREEQYNSTYRVVSVLTVLHQDWLNGKEYKCKVSNKALPAPIEKTISKAKGQPREPQVYTLPPSRDELTKNQVSLSCAVKGFYPSDIAVEWESNGQPENNYKTTPPVLDSDGSFFLVSALTVDKSRWQQGNVFSCSVMHEALHNHYTQKSLSLSPGK

SEQ ID NO: 50 - protein, 471 aa, synthetic construct
  REGION 1..471: note = FC26
EVQLLESGGGVVQPGRSLRLSCIASGFTFSSYPMTWVRQAPGKGLEWVASISYDGSYKYKADSMKGRLTISRDNSKNTLYLEMNSLTAEDTAVYYCARTAFFNAYDFWGQGTLVTVSSASTKGPSVGGGGSGGGGSEIVMTQSPATLSVSPGERATLSCRASQSVRSNLAWYQQKPGQAPRLLIYAASTRATGIPARFSGSGSGTEFTLTISSLQSEDFAVYYCQQYNEWFRTSGQGTKVEIKRDKTHTCPPCPAPELLGGPSVFLFPPKPKDTLMISRTPEVTCVVVDVSHENPEVKFNWYVDGVEVHNAKTKPREEQYNSTYRVVSVLTVLHQDWLNGKEYKCKVSNKALPAPIEKTISKAKGQPREPQVYTLPPSRDELTKNQVSLWCLVKGFYPSDIAVEWESNGQPENNYKTTPPVLSSDGSFKLYSKLTVDKSRWQQGNVFSCSVMHEALHNHYTQKSLSLSPGK

SEQ ID NO: 51 - protein, 227 aa, synthetic construct
  REGION 1..227: note = FC27
DKTHTCPPCPAPELLGGPSVFLFPPKPKDTLMISRTPEVTCVVVDVSHEDPEVKFNWYVDGVEVHNAKTKPREEQYNSTYRVVSVLTVLHQDWLNGKEYKCKVSNKALPAPIEKTISKAKGQPREPQVYTLPPSRDELTKNQVSLSCAVKGFYPSDIAVEWESNGQPENNYDTTPPVLDSDGSFFLVSALTVDKSRWQQGNVFSCSVMHEALHNHYTQKSLSLSPGK

SEQ ID NO: 52 - protein, 227 aa, synthetic construct
  REGION 1..227: note = FC28
DKTHTCPPCPAPELLGGPSVFLFPPKPKDTLMISRTPEVTCVVVDVSHEDPEVKFNWYVDGVEVHNAKTKPREEQYNSTYRVVSVLTVLHQDWLNGKEYKCKVSNKALPAPIEKTISKAKGQPREPQVYTLPPSRDELTKNQVSLSCGVKGFYPSDIAVEWESNGQPENNYKTTPPVLDSDGSFFLASALTVDKSRWQQGNVFSCSVMHEALHNHYTQKSLSLSPGK

SEQ ID NO: 53 - protein, 471 aa, synthetic construct
  REGION 1..471: note = FC29
EVQLLESGGGVVQPGRSLRLSCIASGFTFSSYPMTWVRQAPGKGLEWVASISYDGSYKYKADSMKGRLTISRDNSKNTLYLEMNSLTAEDTAVYYCARTAFFNAYDFWGQGTLVTVSSASTKGPSVGGGGSGGGGSEIVMTQSPATLSVSPGERATLSCRASQSVRSNLAWYQQKPGQAPRLLIYAASTRATGIPARFSGSGSGTEFTLTISSLQSEDFAVYYCQQYNEWFRTSGQGTKVEIKRDKTHTCPPCPAPELLGGPSVFLFPPKPKDTLMISRTPEVTCVVVDVSHENPEVKFNWYVDGVEVHNAKTKPREEQYNSTYRVVSVLTVLHQDWLNGKEYKCKVSNKALPAPIEKTISKAKGQPREPQVDTLPPSRDELTKNQVSLWCLVKGFYPSDIAVEWESNGQPENNYKTTPPVLDSDGSFKLYSKLTVDKSRWQQGNVFSCSVMHEALHNHYTQKSLSLSPGK

SEQ ID NO: 54 - protein, 227 aa, synthetic construct
  REGION 1..227: note = FC30
DKTHTCPPCPAPELLGGPSVFLFPPKPKDTLMISRTPEVTCVVVDVSHEDPEVKFNWYVDGVEVHNAKTKPREEQYNSTYRVVSVLTVLHQDWLNGKEYKCKVSNKALPAPIEKTISKAKGQPREPQVYTLPPSRDALTKNQVSLSCAVKGFYPSDIAVEWESNGQPENNYKTTPPVLDSDGSFFLVSALTVDKSRWQQGNVFSCSVMHEALHNHYTQKSLSLSPGK

SEQ ID NO: 55 - protein, 471 aa, synthetic construct
  REGION 1..471: note = FC31
EVQLLESGGGVVQPGRSLRLSCIASGFTFSSYPMTWVRQAPGKGLEWVASISYDGSYKYKADSMKGRLTISRDNSKNTLYLEMNSLTAEDTAVYYCARTAFFNAYDFWGQGTLVTVSSASTKGPSVGGGGSGGGGSEIVMTQSPATLSVSPGERATLSCRASQSVRSNLAWYQQKPGQAPRLLIYAASTRATGIPARFSGSGSGTEFTLTISSLQSEDFAVYYCQQYNEWFRTSGQGTKVEIKRDKTHTCPPCPAPELLGGPSVFLFPPKPKDTLMISRTPEVTCVVVDVSHENPEVKFNWYVDGVEVHNAKTKPREEQYNSTYRVVSVLTVLHQDWLNGKEYKCKVSNKALPAPIEKTISKAKGQPREPQVDTLPPDRDELTKNQVSLWCLVKGFYPSDIAVEWESNGQPENNYKTTPPVLDSDGSFKLYSKLTVDKSRWQQGNVFSCSVMHEALHNHYTQKSLSLSPGK

SEQ ID NO: 56 - protein, 227 aa, synthetic construct
  REGION 1..227: note = FC 32
DKTHTCPPCPAPELLGGPSVFLFPPKPKDTLMISRTPEVTCVVVDVSHEDPEVKFNWYVDGVEVHNAKTKPREEQYNSTYRVVSVLTVLHQDWLNGKEYKCKVSNKALPAPIEKTISKAKGQPREPQVYTLPPSRDELTKNQVSLWCLVKGFYPSDIAVEWESNGQPENNYKTTPPVLDSDGSFFLYSALTVDKSRWQQGNVFSCSVMHEALHNHYTQKSLSLSPGK

SEQ ID NO: 57 - protein, 227 aa, synthetic construct
  REGION 1..227: note = FC 33
DKTHTCPPCPAPELLGGPSVFLFPPKPKDTLMISRTPEVTCVVVDVSHEDPEVKFNWYVDGVEVHNAKTKPREEQYNSTYRVVSVLTVLHQDWLNGKEYKCKVSNKALPAPIEKTISKAKGQPREPQVYTLPPSRDELTKNQVSLSCAVKGFYPSDIAVEWESNGQPENNYKTTPPVLDSDGSFKLVSKLTVDKSRWQQGNVFSCSVMHEALHNHYTQKSLSLSPGK